European Patent Specification EP 3 530 670 B1, published February 28, 2024. Title: Recombinant protein of Limulus and cDNA encoding the same. Applicant: Seikagaku Corporation. The sequence listing filed with the application follows.

SEQUENCE LISTING (34 sequences)

SEQ ID NO: 1 - DNA, 3063 bp, Limulus polyphemus
atggtactagcgtcgttcttggtgtctggtttagttctagggctattagcccaacaaatgcacccagttcagtccagaggagtagatctgggcttgtgtgatgacacgaggtttgagtgtaagtgtggagatccaggatacgtgttcaacgtccccgcgaagcaatgtacgtacttctatcgatggaggccttattgtaaaccatgtgacaaactggaggctaaagatgtgtgtcccaagtacaaacgatgtcaagagtgtagggctggtctcgacagttgtgtgagttgtccacctaacaaatatggaacttggtgtagcggtgagtgtcagtgtaagaatgggggtatttgtgatcagaggacaggagcttgtacatgtcgtgacagatatgaaggtgtgcattgtgaaatccttcaaggttgtcctcttcttcaatcggatccccaggttcaggaagtaaaaaatccaccaaatgatccacaaactattgactacagctgttcaccaggcttcaagcttaaaggcgtggcacgtatcacctgtcttccaaatgggcagtggagtagctttccacccaaatgtattcgagaatgttccatggtttcatctctagaacatggcaaagtaaactctcctagtgccgatctgatagaaggagctactttaaggttctcatgtgatagtccctactacttgattggtcaagaaacattaacctgccagggcaacggtcagtggagtgggcagataccacagtgtcagaaattggtcttctgccctgaccttgaccctgtaagccatgctgaacaccaggttaaaattggcctagaacaaaaatatggtcaatttcctcaaggcactgaagtaacctatacgtgtactggtaattacttcttgatgggtttggacaccttaaaatgtaaccctgatgggtcctggtcgggaacacagccgtcctgtgttaaagtggcagacagagaggtcaactgtgacagtaaagctgtggacttcttggatgatgttggcgaacctgtcaggatccactgtcctgctggctgttccttaactgctggtactgtatggggtacagccatatatcacgaactttcctcagtatgtcgtgcagctattcatgctggcaaggttccaaactctggaggtgcagtgcatgtagtgaacaacggtccgtactcagactttctggctagtgatctgaatgggataaaatcagacgagttgaagtctcttgctcagagtttccgattcgattatgtcagttcatcaacagcagggagaaagtcaggatgtcctgatggatggttcgagattgaggagaactgtgtgtacgttacatcgaaacagagagcctgggaaagagctcaaggtgtatgtaccaatatggccgctcgtcttgctgtgttagacaaagatgtaattccaagttccttgactgagactctacgagggaaagggttagcaacgacgtggattggactacacagattagatgctgataatcactttatttgggagctaatggatcgcagtagtgttgctttgaatgacagcctaacattctgggctcctggagaacctgggaatgaaactaactgtgtatatctggatatccaagatcagctacagccagtgtggaaaaccaagtcttgttttcaaccctcaagttttgtttgtatgatggatttgtcagacaagaacaaagccaaatgcaaagaccctggacctttggaaaacggacacgccaagcttcatggtcaaagtattgatggattttatgctgggtcttctgtaagatacagctgcgaggtcctccactacctcagtggaactgagacagtatcttgtacatcaaatggcacgtggagtgcccctaaacctcgatgtattaaagtcatcacctgccaaacccctcctgtaccatcctatggttctgtggacatcaaacccccaagtagaacaaactcaatcagtcgtgttgggtcgccattcttgaggttgccacggttacccctccctttagccagagcagccggacctcctccaaaacctagatccgcaccaccctctactgtggacctgtcttccaaggtcaaactgcctgaaggtcattaccgggtggggtctcaagccatttacacgtgcgagtcaagatactacgaactgcttggatctcaaggtagaagatgcgactctaatggaaagtggagtggtcgaccagcaagctgtataccagtttgtggacggtcagactctccccgttctcctttcatcgtcaatggaaattccaccgaaataggtcagtggccgtggcaggcaggaatctccagatggcttgcagatcataatatgtggtttcttcagtgtggaggagctctactgaatgagaaatggatcattactgcagcccactgtgtcacctactctgctactgccgagatcattgacccaagtcagtttaaattctacctgggcaaatactatcgagatgacagtaaggatgatgactacgtacaagtaagagaggctatcgagatccatgtgaatcctaactacgatcctggaaatctcaactttgacatagccctgattcaactgaagacttctgttgctctgaccacacgagtgcaaccaatatgtctgcctactgatctcactacaagagaaaacctgaaagagggagcgttagcggtggtgacaggatggggtttgaatgaaaacaacacatattcagagatgattcagcaagccgttctgcctgttgttgcagcaagcacctgtgaacaaggatatcaggactcgggcttgccactgacagtgacagagaacatgttctgtgcaggttacaagcaggggcgctatgatgcctgcagtggagacagtggaggaccattagtgtttgctgatgattcccgcaccgataggcggtgggtcctggaagggatcgtcagctggggcagccccaatggatgtggcaagtctaaccagtatgggggcttcactaaagttaacgtttttctatcgtggattcggcagttcatttga

SEQ ID NO: 2 - protein, 1020 aa, Limulus polyphemus
MVLASFLVSGLVLGLLAQQMHPVQSRGVDLGLCDDTRFECKCGDPGYVFNVPAKQCTYFYRWRPYCKPCDKLEAKDVCPKYKRCQECRAGLDSCVSCPPNKYGTWCSGECQCKNGGICDQRTGACTCRDRYEGVHCEILQGCPLLQSDPQVQEVKNPPNDPQTIDYSCSPGFKLKGVARITCLPNGQWSSFPPKCIRECSMVSSLEHGKVNSPSADLIEGATLRFSCDSPYYLIGQETLTCQGNGQWSGQIPQCQKLVFCPDLDPVSHAEHQVKIGLEQKYGQFPQGTEVTYTCTGNYFLMGLDTLKCNPDGSWSGTQPSCVKVADREVNCDSKAVDFLDDVGEPVRIHCPAGCSLTAGTVWGTAIYHELSSVCRAAIHAGKVPNSGGAVHVVNNGPYSDFLASDLNGIKSDELKSLAQSFRFDYVSSSTAGRKSGCPDGWFEIEENCVYVTSKQRAWERAQGVCTNMAARLAVLDKDVIPSSLTETLRGKGLATTWIGLHRLDADNHFIWELMDRSSVALNDSLTFWAPGEPGNETNCVYLDIQDQLQPVWKTKSCFQPSSFVCMMDLSDKNKAKCKDPGPLENGHAKLHGQSIDGFYAGSSVRYSCEVLHYLSGTETVSCTSNGTWSAPKPRCIKVITCQTPPVPSYGSVDIKPPSRTNSISRVGSPFLRLPRLPLPLARAAGPPPKPRSAPPSTVDLSSKVKLPEGHYRVGSQAIYTCESRYYELLGSQGRRCDSNGKWSGRPASCIPVCGRSDSPRSPFIVNGNSTEIGQWPWQAGISRWLADHNMWFLQCGGALLNEKWIITAAHCVTYSATAEIIDPSQFKFYLGKYYRDDSKDDDYVQVREAIEIHVNPNYDPGNLNFDIALIQLKTSVALTTRVQPICLPTDLTTRENLKEGALAVVTGWGLNENNTYSEMIQQAVLPVVAASTCEQGYQDSGLPLTVTENMFCAGYKQGRYDACSGDSGGPLVFADDSRTDRRWVLEGIVSWGSPNGCGKSNQYGGFTKVNVFLSWIRQFI

SEQ ID NO: 3 - DNA, 3063 bp, Limulus polyphemus
atggtactagcgtcgttcttggtgtctggtttagttctagggctattagcccaacaaatgcacccagttcagtccagaggagtagatctgggcttgtgtgatgacacgaggtttgagtgtaagtgtggagatccaggatacgtgttcaacgtccccgcgaagcaatgtacgtacttctatcgatggaggccttattgtaaaccatgtgacaaactggaggctaaagatgtgtgtcccaagtacaaacgatgtcaagagtgtagggctggtctcgacagttgtgtgagttgtccacctaacaaatatggaacttggtgtagcggtgagtgtcagtgtaagaatgggggtatttgtgatcagaggacaggagcttgtacatgtcgtgacagatatgaaggtgtgcattgtgaaatccttcaaggttgtcctcttcttcaatcggatccccaggttcaggaagtaaaaaatccaccaaatgatccacaaactattgactacagctgttcaccaggcttcaagcttaaaggcgtggcacgtatcacctgtcttccaaatgggcagtggagtagctttccacccaaatgtattcgagaatgttccatggtttcatctctagaacatggcaaagtaaactctcctagtgccgatctgatagaaggagctactttaaggttctcatgtgatagtccctactacttgattggtcaagaaacattaacctgccagggcaacggtcagtggagtgggcagataccacagtgtcagaaattggtcttctgccctgaccttgaccctgcaagccatgctgaacaccaggttaaaattggcctagaacaaaaatatggtcaatttcctcaaggcactgaagtaacctatacgtgtactggtaattacttcttgatgggtttggacaccttaaaatgtaaccctgatgggtcctggtcgggaacacagccgtcctgtgttaaagtggcagacagagaggtcaactgtgacagtaaagctgtggacttcttggatgatgttggcgaacctgtcaggatccactgtcctgctggctgttccttaactgctggtactgtatggggtacagccatatatcacgaactttcctcagtatgtcgtgcagctattcatgctggcaaggttccaaactctggaggtgcagtgcatgtagtgaacaacggtccgtactcagactttctggctagtgatctgaatgggataaaatcagacgagttgaagtctcttgctcagagtttccgattcgattatgtcagttcatcaacagcagggagaaagtcaggatgtcctgatggatggttcgagattgaggagaactgtgtgtacgttacatcgaaacagagagcctgggaaagagctcaaggtgtatgtaccaatatggccgctcgtcttgctgtgttagacaaagatgtaattccaagttccttgactgagactctacgagggaaagggttagcaacgacgtggattggactacacagattagatgctgataatcactttatttgggagctaatggatcgcagtagtgttgctttgaatgacagcctaacattctgggctcctggagaacctgggaatgaaactaactgtgtatatctggatatccaagatcagctacagccagtgtggaaaaccaagtcttgttttcaaccctcaagttttgtttgtatgatggatttgtcagacaagaacaaagccaaatgcaaagaccctggacctttggaaaacggacacgccaagcttcatggtcaaagtattgatggattttatgctgggtcttctgtaagatacagctgcgaggtcctccactacctcagtggaactgagacagtatcttgtacatcaaatggcacgtggagtgcccctaaacctcgatgtattaaagtcatcacctgccaaacccctcctgtaccatcctatggttctgtggacatcaaacccccaagtagaacaaactcaatcagtcgtgttgggtcgccattcttgaggttgccacggttacccctccctttagccagagcagccggacctcctccaaaacctagatccgcaccaccctctactgtggacctgtcttccaaggtcaaactgcctgaaggtcattaccgggtggggtctcaagccatttacacgtgcgagtcaagatactacgaactgcttggatctcaaggtagaagatgcgactctaatggaaagtggagtggtcgaccagcaagctgtataccagtttgtggacggtcagactctccccgttctcctttcatcgtcaatggaaattccaccgaaataggtcagtggccgtggcaggcaggaatctccagatggcttgcagatcataatatgtggtttcttcagtgtggaggagctctactgaatgagaaatggatcattactgcagcccactgtgtcacctactctgctactgccgagatcattgacccaagtcagtttaaattctacctgggcaaatactatcgagatgacagtaaggatgatgactacgtacaagtaagagaggctatcgagatccatgtgaatcctaactacgatcctggaaatctcaactttgacatagccctgattcaactgaagacttctgttgctctgaccacacgagtgcaaccaatatgtctgcctactgatctcactacaagagaaaacctgaaagagggagcgttagcggtggtgacaggatggggtttgaatgaaaacaacacatattcagagatgattcagcaagccgttctgcctgttgttgcagcaagcacctgtgaacaaggatatcaggactcgggcttgccactgacagtgacagagaacatgttctgtgcaggttacaagcaggggcgctatgatgcctgcagtggagacagtggaggaccattagtgtttgctgatgattcccgcaccgataggcggtgggtcctggaagggatcgtcagctggggcagccccaatggatgtggcaagtctaaccagtatgggggcttcactaaagttaacgtttttctatcgtggattcggcagttcatttga

SEQ ID NO: 4 - protein, 1020 aa, Limulus polyphemus
MVLASFLVSGLVLGLLAQQMHPVQSRGVDLGLCDDTRFECKCGDPGYVFNVPAKQCTYFYRWRPYCKPCDKLEAKDVCPKYKRCQECRAGLDSCVSCPPNKYGTWCSGECQCKNGGICDQRTGACTCRDRYEGVHCEILQGCPLLQSDPQVQEVKNPPNDPQTIDYSCSPGFKLKGVARITCLPNGQWSSFPPKCIRECSMVSSLEHGKVNSPSADLIEGATLRFSCDSPYYLIGQETLTCQGNGQWSGQIPQCQKLVFCPDLDPASHAEHQVKIGLEQKYGQFPQGTEVTYTCTGNYFLMGLDTLKCNPDGSWSGTQPSCVKVADREVNCDSKAVDFLDDVGEPVRIHCPAGCSLTAGTVWGTAIYHELSSVCRAAIHAGKVPNSGGAVHVVNNGPYSDFLASDLNGIKSDELKSLAQSFRFDYVSSSTAGRKSGCPDGWFEIEENCVYVTSKQRAWERAQGVCTNMAARLAVLDKDVIPSSLTETLRGKGLATTWIGLHRLDADNHFIWELMDRSSVALNDSLTFWAPGEPGNETNCVYLDIQDQLQPVWKTKSCFQPSSFVCMMDLSDKNKAKCKDPGPLENGHAKLHGQSIDGFYAGSSVRYSCEVLHYLSGTETVSCTSNGTWSAPKPRCIKVITCQTPPVPSYGSVDIKPPSRTNSISRVGSPFLRLPRLPLPLARAAGPPPKPRSAPPSTVDLSSKVKLPEGHYRVGSQAIYTCESRYYELLGSQGRRCDSNGKWSGRPASCIPVCGRSDSPRSPFIVNGNSTEIGQWPWQAGISRWLADHNMWFLQCGGALLNEKWIITAAHCVTYSATAEIIDPSQFKFYLGKYYRDDSKDDDYVQVREAIEIHVNPNYDPGNLNFDIALIQLKTSVALTTRVQPICLPTDLTTRENLKEGALAVVTGWGLNENNTYSEMIQQAVLPVVAASTCEQGYQDSGLPLTVTENMFCAGYKQGRYDACSGDSGGPLVFADDSRTDRRWVLEGIVSWGSPNGCGKSNQYGGFTKVNVFLSWIRQFI

SEQ ID NO: 5 - DNA, 1203 bp, Limulus polyphemus
atggcgtggatttgtgtgataacgttgtttgctttggcttctagtacgttgagtaataaagttagtagagtggggatcatctttcctaagacacagaacgataataaacagtgtacagcaaaaggtggattaaaagggtcctgcaagtccctcacagactgtcctgctgtcttggctacgttgaaggatagtttccctgtcgtttgctcttggaatggtcggtttcagcctattgtatgttgtcctgatgcagcagcaccaagtgtaaccacaacagttacaactattgtccctacaaaagaaacaaagattccaagattacatataccaggttgtggaaaaagaaaagtaaatgtagatattacaactattggacgttcggggtcaccaatacttcctcccatatctacttctcaagatttgaagggtgggagaggaatcattgctggaggtgtagaagctaaaattggcgcctggccttggatggcagctgtttttgtgaaaaattttggcattggcagattccattgtgctggtagcataatcagtagcaagtacattttgtctgctgcccacgctttcctcattggaggtcgaaagctgaccccaactcgcttagctgtccgcgtaggaggccactacgtaaagatgggtcaagaatatcatgtggaagatgtgattatccatcctgactacgtagaaagggagaattacaatgatattgctatcattgtgttaaaagaggaactgaattttactgatttggtccgtccaatctgtctccctgacccagaggcagtaacagattcattaaaaggcagaagggtgacagtagctggatggggtgatctggatttcgccggtccacgaagtcaagttctgcgcgaggttagtatccccgttgttccaatcggtgactgtaacaaagcctatcagaagctcaacacccttgctcttaaaaatgggataacgaaaaagtttatttgtgctggattggaagaaggtgggaaagatgcttgtcaaggcgattctggtggaccgttgatgctagtgaacaatagtagttggatagtgacgggagtggtgtcgttcggacacaagtgtgccgaggagggatttcctggtgtgtacacgcgtgtagtgagttacctagagtggatcgcgaaggttacgaactcgttagaccaggcagtcactaactga

SEQ ID NO: 6 - protein, 400 aa, Limulus polyphemus
MAWICVITLFALASSTLSNKVSRVGIIFPKTQNDNKQCTAKGGLKGSCKSLTDCPAVLATLKDSFPVVCSWNGRFQPIVCCPDAAAPSVTTTVTTIVPTKETKIPRLHIPGCGKRKVNVDITTIGRSGSPILPPISTSQDLKGGRGIIAGGVEAKIGAWPWMAAVFVKNFGIGRFHCAGSIISSKYILSAAHAFLIGGRKLTPTRLAVRVGGHYVKMGQEYHVEDVIIHPDYVERENYNDIAIIVLKEELNFTDLVRPICLPDPEAVTDSLKGRRVTVAGWGDLDFAGPRSQVLREVSIPVVPIGDCNKAYQKLNTLALKNGITKKFICAGLEEGGKDACQGDSGGPLMLVNNSSWIVTGVVSFGHKCAEEGFPGVYTRVVSYLEWIAKVTNSLDQAVTN

SEQ ID NO: 7 - DNA, 1203 bp, Limulus polyphemus
atggcgtggatttgtgtgataacgttgtttgctttggcttctagtacgttgagtaataaagttagtagagtggggatcatctttcctaagacacagaacgataataaacagtgtacagcaaaaggtggattaaaagggtcctgcaagtccctcacagactgtcctgctgtcttggctacgttgaaggatagtttccctgtcgtttgctcttggaatggtcggtttcagcctattgtatgttgtcctgatgcagcagcaccaagtgtaaccacaacagttacaactattgtccctacaaaagaaacaaagattccaagattacatataccaggttgtggaaaaagaaaagtaaatgtagatattacaactattggacgttcggggtcaccaatacttcctcccatatctacttctcaagatttgaagggtgggagaggaatcattgctggaggtgtagaagctaaaattggcgcctggccttggatggcagctgtttttgtgaaaaattttggcattggcagattccattgtgctggtagcataatcagtagcaagtacattttgtctgctgcccacgctttcctcattggaggtcgaaagctgaccccaactcgcttagctgtccgcgtaggaggccactacgtaaagatgggtcaagaatatcatgtggaagatgtgattatccatcctgactacgtagaaagggagaattacaatgatattgctatcattgtgttaaaagaggaactgaattttactgatttggtccgtccaatctgtctccctgacccagaggcagtaacagattcattaaaaggcagaagggtgacagtagctggatggggtgatctggatttcgccggtccacgaagtcaagttctgcgcgaggttagtatccccgttgttccaatcagtgattgtaacaaagcctatcagaatctcaacacccttgctcttaaaaatgggataacgaaaaagtttatttgtgctggattggaagaaggtgggaaagatgcttgtcaaggcgattctggtggaccgttgatgctagtgaacaatagtagttggatagtgacgggagtggtgtcgttcggacacaagtgtgccgaggagggatttcctggtgtgtacacgcgtgtagtgagttacctagagtggatcgcgaaggttacgaactcgttagaccaggcagtcactaactga

SEQ ID NO: 8 - protein, 400 aa, Limulus polyphemus
MAWICVITLFALASSTLSNKVSRVGIIFPKTQNDNKQCTAKGGLKGSCKSLTDCPAVLATLKDSFPVVCSWNGRFQPIVCCPDAAAPSVTTTVTTIVPTKETKIPRLHIPGCGKRKVNVDITTIGRSGSPILPPISTSQDLKGGRGIIAGGVEAKIGAWPWMAAVFVKNFGIGRFHCAGSIISSKYILSAAHAFLIGGRKLTPTRLAVRVGGHYVKMGQEYHVEDVIIHPDYVERENYNDIAIIVLKEELNFTDLVRPICLPDPEAVTDSLKGRRVTVAGWGDLDFAGPRSQVLREVSIPVVPISDCNKAYQNLNTLALKNGITKKFICAGLEEGGKDACQGDSGGPLMLVNNSSWIVTGVVSFGHKCAEEGFPGVYTRVVSYLEWIAKVTNSLDQAVTN

SEQ ID NO: 9 - DNA, 1203 bp, Limulus polyphemus
atggcgtggatttgtgtgataacgttgtttgctttggcttctagtacgttgagtaataaagttagtagagtggggatcatctttcctaagacacagaacgataataaacagtgtacagcaaaaggtggattaaaagggtcctgcaagtccctcacagactgtcctgctgtcttggctacgttgaaggatagtttccctgtcgtttgctcttggaatggtcggtttcagcctattgtatgttgtcctgatgcagcagcaccaagtgtaaccacaacagttacaactattgtccctacaaaagaaacaaagattccaagattacatataccaggttgtggaaaaagaaaagtaaatgtagatattacaactattggacgttcggggtcaccaatacttcctcccatatctacttctcaagatttgaagggtgggagaggaatcattgctggaggtgtagaagctaaaattggcgcctggccttggatggcagctgtttttgtgaaaaattttggcattggcagattccattgtgctggtagcataatcagtagcaagtacattttgtctgctgcccacgctttcctcattggaggtcgaaagctgaccccaactcgcttagctgtccgcgtaggaggccactacgtaaagatgggtcaagaatatcatgtggaagatgtgattatccatcctgactacgtagaaagggagaattacaatgatattgctatcattgtgttaaaagaggaactgaattttactgatttggtccgtccaatctgtctccctgacccagaggcagtaacagattcattaaaaggcagaagggtgacagtagctggatggggtgatctggatttcgccggtccacgaagtcaagttctgcgcgaggttagtatccccgttgttccaatcagtgattgtaacaaagcctatcagaatctcaacacccttgctcttaaaaatgggataacgaacaagtttatttgtgctggattggaagaaggcgggaaagatgcttgtcaaggcgattctggtggaccgttgatgctagtgaacaatagtagttggatagtgacgggagtggtgtcgttcggacacaagtgtgccgaggagggatttcctggtgtgtacacgcgtgtagtgagttacctagagtggatcgcgaaggttacgaactcgttagaccaggcagtcactaactga

SEQ ID NO: 10 - protein, 400 aa, Limulus polyphemus
MAWICVITLFALASSTLSNKVSRVGIIFPKTQNDNKQCTAKGGLKGSCKSLTDCPAVLATLKDSFPVVCSWNGRFQPIVCCPDAAAPSVTTTVTTIVPTKETKIPRLHIPGCGKRKVNVDITTIGRSGSPILPPISTSQDLKGGRGIIAGGVEAKIGAWPWMAAVFVKNFGIGRFHCAGSIISSKYILSAAHAFLIGGRKLTPTRLAVRVGGHYVKMGQEYHVEDVIIHPDYVERENYNDIAIIVLKEELNFTDLVRPICLPDPEAVTDSLKGRRVTVAGWGDLDFAGPRSQVLREVSIPVVPISDCNKAYQNLNTLALKNGITNKFICAGLEEGGKDACQGDSGGPLMLVNNSSWIVTGVVSFGHKCAEEGFPGVYTRVVSYLEWIAKVTNSLDQAVTN

SEQ ID NO: 11 - DNA, 1203 bp, Limulus polyphemus
atggcgtggatttgtgtgataacgttgtttgctttggcttctagtacgttgagtaataaagttagtagagtggggatcatctttcctaagacacagaacgataataaacagtgtacagcaaaaggtggattaaaagggtcctgcaagtccctcacagactgtcctgctgtcttggctacgttgaaggatagtttccctgtcgtttgctcttggaatggtcggtttcagcctattgtatgttgtcctgatgcagcagcaccaagtgtaaccacaacagttacaactattgtccctacaaaagaaacaaagattccaagattacatataccaggttgtggaaaaagaaaagtaaatgtagatattacaactattggacgttcggggtcaccaatacttcctcccatatctacttctcaagatttgaagggtgggagaggaatcattgctggaggtgtagaagctaaaattggcgcctggccttggatggcagctgtttttgtgaaaaattttggcattggcagatttcattgtgctggtagcataatcagtagcaagtacattttgtctgctgcccacgctttcctcattggaggtcgaaagctgaccccaactcgcttagctgtccgcgtaggaggccactacgtaaagatgggtcaagaatatcatgtggaagatgtgattatccatcctgactacgtagaaagggagaattacaatgatattgctatcattgtgttaaaagaggaactgaattttactgatttggtccgtccaatctgtctccctgacccagaggcagtaacagattcattaaaaggcagaagggtgacagtagctggatggggtgatctggatttcgccggtccacgaagtcaagttctgcgcgaggttagtatccccgttgttccaatcagtgattgtaacaaagcctatcagaatctcaacacccttgctcttaaaaatgggataacgaacaagtttatttgtgctggattggaagaaggcgggaaagatgcttgtcaaggcgattctggtggaccgttgatgctagtgaacaatagtagttggatagtgacgggagtggtgtcgttcggacacaagtgtgccgaggagggatttcctggtgtgtacacgcgtgtagtgagttacctagagtggatcgcgaaggttacgaactcgttagaccaggcagtcactaagtga

SEQ ID NO: 12 - protein, 400 aa, Limulus polyphemus
MAWICVITLFALASSTLSNKVSRVGIIFPKTQNDNKQCTAKGGLKGSCKSLTDCPAVLATLKDSFPVVCSWNGRFQPIVCCPDAAAPSVTTTVTTIVPTKETKIPRLHIPGCGKRKVNVDITTIGRSGSPILPPISTSQDLKGGRGIIAGGVEAKIGAWPWMAAVFVKNFGIGRFHCAGSIISSKYILSAAHAFLIGGRKLTPTRLAVRVGGHYVKMGQEYHVEDVIIHPDYVERENYNDIAIIVLKEELNFTDLVRPICLPDPEAVTDSLKGRRVTVAGWGDLDFAGPRSQVLREVSIPVVPISDCNKAYQNLNTLALKNGITNKFICAGLEEGGKDACQGDSGGPLMLVNNSSWIVTGVVSFGHKCAEEGFPGVYTRVVSYLEWIAKVTNSLDQAVTK

SEQ ID NO: 13 - DNA, 1128 bp, Limulus polyphemus
atgttggtgaataacatgttttcattgctgtgtttcccactcctgatgtctatgtttagctgcagtagtctcggcagacagcgtagacagtttgttttccccgatgatgaagaatcatgctcaaaccgatttactaacgatggaatatgtaaagatgttttgaattgtagagatcttttacaaaaaaatgattataatttactgaaagaatcaatatgcggttttgaaggcataacacccaaagtttgttgtccgaaacaaagtattgtaaatccaataacagaagcacctccaaaaaccactacaactgaacgaccgccaatacggataccatccaatcttcctaaacagtgtggaaatcgtaatattacaactaccaggattattggagggcaggaagcaacacctggagcctggccctggatggctgctgtctatatcaaacaaggaggaatcagaagtgttcagtgtggaggtgcgcttgtcaccaacaggcacgtgattacagcatcgcactgtgttgtaaacagtttaggaacagatgtgatgcgagctgacgtattctcggttcgcctaggtgaacacaatttatatagcaccaatgacagttcagatccaattgattttgcagttacgtcagtgaaacatcatgaaaactttgtgctcgcgacgtatttgaatgatatcgcaattctgaagttaaacgacactgttacgtttacgcacaaaattaaaccaatttgtctaccttatgaaagcttaaggtatgaggatctagcaatgagaaacccatttgtcgccggatggggaacaacagcatttaatggcccatctagtgcagtattacgagaagtgcagttaccaatatggggacacgagccctgcaggcaggcctacgagaaggatttaaatattacaaacgtgtatatgtgtgctgggtatgcagatggcggtaaagatgcttgccagggtgattctggaggtccaatgatgttgcctgataaaagcgggaacttttatctcgttggaattgtgtctttcggaaagaaatgcgcgttgcctggatttcctggggtttacacaaaagtgaccgaatttttagattggattgcagtaaatatggtgtag

SEQ ID NO: 14 - protein, 375 aa, Limulus polyphemus
MLVNNMFSLLCFPLLMSMFSCSSLGRQRRQFVFPDDEESCSNRFTNDGICKDVLNCRDLLQKNDYNLLKESICGFEGITPKVCCPKQSIVNPITEAPPKTTTTERPPIRIPSNLPKQCGNRNITTTRIIGGQEATPGAWPWMAAVYIKQGGIRSVQCGGALVTNRHVITASHCVVNSLGTDVMRADVFSVRLGEHNLYSTNDSSDPIDFAVTSVKHHENFVLATYLNDIAILKLNDTVTFTHKIKPICLPYESLRYEDLAMRNPFVAGWGTTAFNGPSSAVLREVQLPIWGHEPCRQAYEKDLNITNVYMCAGYADGGKDACQGDSGGPMMLPDKSGNFYLVGIVSFGKKCALPGFPGVYTKVTEFLDWIAVNMV

SEQ ID NO: 15 - DNA, 1128 bp, Limulus polyphemus
atgttggtgaataacatgttttcattgctgtgtttcccactcctgatgtctatgtttagctgcagtagtctcggcagacagcgtagacagtttgttttccccgatgatgaagaatcatgctcaaaccgatttactaacgatggaatatgtaaagatgttttgaattgtagagatcttttacaaaaaaatgattataatttactgaaagaatcaatatgcggttttgaaggcataacacccaaagtttgttgtccgaaacaaagtattgtaaatccaataacagaagcacctccaaaaaccactacaactgaacgaccgccaatacggataccatccaatcttcctaaacagtgtggaaatcgtaatattacaactaccaggattattggagggcaggaagcaacacctggagcctggccctggatggctgctgtctatatcaaacaaggaggaatcagaagtgctcagtgtggaggtgcgcttgtcaccaacaggcacgtgattacagcatcgcactgtgttgtaaacagtttaggaacagatgtgatgcgagctgatgtattctcggttcgcctaggtgaacacaatttatatagcaccaatgacagttcagatccaattgattttgcagttacgtcagtgaaacatcatgaaaactttgtgctcgcgacgtatttgaatgatatcgcaattctgaagttaaacgacactgttacgtttacgcacaaaattaaaccaatttgtctaccttatgaaagcttaaggtatgaggatctagcaatgagaaacccatttgtcgccggatggggaacaacagcatttaatggcccatctagtgcagtattacgagaagtgcagttaccaatatggggacacgagccctgcaggcaggcctacgagaaggatttaaatattacaaacgtgtatatgtgtgctgggtatgcagatggcggtaaagatgcttgccagggtgattctggaggtccaatgatgttgcctgataaaagcgggaacttttatctcgttggaattgtgtctttcggaaagaaatgcgcgttgcctggatttcctggggtttacacaaaagtgaccgaatttttagattggattgcagtaaatatggtgtag

SEQ ID NO: 16 - protein, 375 aa, Limulus polyphemus
MLVNNMFSLLCFPLLMSMFSCSSLGRQRRQFVFPDDEESCSNRFTNDGICKDVLNCRDLLQKNDYNLLKESICGFEGITPKVCCPKQSIVNPITEAPPKTTTTERPPIRIPSNLPKQCGNRNITTTRIIGGQEATPGAWPWMAAVYIKQGGIRSAQCGGALVTNRHVITASHCVVNSLGTDVMRADVFSVRLGEHNLYSTNDSSDPIDFAVTSVKHHENFVLATYLNDIAILKLNDTVTFTHKIKPICLPYESLRYEDLAMRNPFVAGWGTTAFNGPSSAVLREVQLPIWGHEPCRQAYEKDLNITNVYMCAGYADGGKDACQGDSGGPMMLPDKSGNFYLVGIVSFGKKCALPGFPGVYTKVTEFLDWIAVNMV

SEQ ID NO: 17 - DNA, 1128 bp, Limulus polyphemus
atgttggtgaataacatgttttcattgctgtgtttcccactcctgatgtctatgtttagctgcagtagtctcggcagacagcgtagacaatttgttttccccgatgatgaagaatcatgctcaaaccgatttactaacgaaggaatatgtaaagatgttttgaattgtagagaacttttacaaaaaaatgattataatttactgaaagaatcaatatgcggttttgaaggcataacacccaaagtttgttgtccgaaacaaagtattgtaaatccaataacagaagcacctccaaaaactactacaactgaacgaccgccaatccgtataccatccaatcttcctaaacagtgtggaaatcgtaatattacaactaccaggattattggagggcaggaagcaacacctggagcctggccctggatggctgctgtctatatcaaacaaggaggaatcagaagtgttcagtgtggaggtgcgcttgtcaccaacaggcacgtgattacagcatcgcactgtgttgtaaacagtttaggaacagatgtgatgcgagctgacgtattctcggttcgcctaggtgaacacaatttatatagcaccaatgacagttcagatccaattgattttgcagttacgtcagtgaaacatcatgaaaactttgtgctcgcgacgtatttgaatgatatcgcaattctgaagttaaacgacactgttacgtttacgcacaaaattaaaccaatttgtctaccttatgaaagcttaaggtatgaggatctagcaatgagaaacccatttgtcgccggatggggaacaacagcatttaatggcccatctagtgcagtattacgagaagtgcagttaccaatatggggacacgagccctgcaggcaggcctacgagaaggatttaaatattacaaacgtgtatatgtgtgctgggtatgcagatggcggtaaagatgcttgccagggtgattctggaggtccaatgatgttgcctgataaaagcgggaacttttatctcgttggaattgtgtctttcggaaagaaatgcgcgttgcctggatttcctggggtttacacaaaagtgaccgaatttttagattggattgcagtaaatatggtgtag

SEQ ID NO: 18 - protein, 375 aa, Limulus polyphemus
MLVNNMFSLLCFPLLMSMFSCSSLGRQRRQFVFPDDEESCSNRFTNEGICKDVLNCRELLQKNDYNLLKESICGFEGITPKVCCPKQSIVNPITEAPPKTTTTERPPIRIPSNLPKQCGNRNITTTRIIGGQEATPGAWPWMAAVYIKQGGIRSVQCGGALVTNRHVITASHCVVNSLGTDVMRADVFSVRLGEHNLYSTNDSSDPIDFAVTSVKHHENFVLATYLNDIAILKLNDTVTFTHKIKPICLPYESLRYEDLAMRNPFVAGWGTTAFNGPSSAVLREVQLPIWGHEPCRQAYEKDLNITNVYMCAGYADGGKDACQGDSGGPMMLPDKSGNFYLVGIVSFGKKCALPGFPGVYTKVTEFLDWIAVNMV

SEQ ID NO: 19 - DNA, 1128 bp, Limulus polyphemus
atgttggtgaataacatgttttcattgctgtgtttcccactcctgatgtctatgtttagctgcagtagtctcggcagacagcgtagacaatttgttttccccgatgatgaagaatcatgctcaaaccgatttactaacgatggaatatgtaaagatgttttgaattgtagagatcttttacaaaaaaatgattataatttactgaaagaatcaatatgcggttttgaaggcataacacccaaagtttgttgtccgaaacaaagtattgtaaatccaataacagaagcacctccaaaaaatactacaactgaacgaccgccaatccgtataccatccaatcttcctaaacagtgtggaaatcgtaatattacaactaccaggattattggagggcaggaagcaacacctggagcctggccctggatggctgctgtctatatcaaacaaggaggaatcagaagtgttcagtgtggaggtgcgcttgtcaccaacaggcacgtgattacagcatcgcactgtgttgtaaacagtttaggaacagatgtgatgcgagctgacgtattctcggttcgcctaggtgaacacaatttatatagcaccaatgacagttcagatccaattgattttgcagttacgtcagtgaaacatcatgaaaactttgtgctcgcgacgtatttgaatgatatcgcaattctgaagttaaacgacactgttacgtttacgcacaaaattaaaccaatttgtctaccttatgaaagcttaaggtatgaggatctagcaatgagaaacccatttgtcgccggatggggaacaacagcatttaatggcccatctagtgcagtattacgagaagtgcagttaccaatatggggacacgagccctgcaggcaggcctacgagaaggatttaaatattacaaacgtgtatatgtgtgctgggtatgcagatggcggtaaagatgcttgccagggtgattctggaggtccaatgatgttgcctgataaaagcgggaacttttatctcgttggaattgtgtctttcggaaagaaatgcgcgttgcctggatttcctggggtttacacaaaagtgaccgaatttttagattggattgcagtaaatatggtgtag

SEQ ID NO: 20 - protein, 375 aa, Limulus polyphemus
MLVNNMFSLLCFPLLMSMFSCSSLGRQRRQFVFPDDEESCSNRFTNDGICKDVLNCRDLLQKNDYNLLKESICGFEGITPKVCCPKQSIVNPITEAPPKNTTTERPPIRIPSNLPKQCGNRNITTTRIIGGQEATPGAWPWMAAVYIKQGGIRSVQCGGALVTNRHVITASHCVVNSLGTDVMRADVFSVRLGEHNLYSTNDSSDPIDFAVTSVKHHENFVLATYLNDIAILKLNDTVTFTHKIKPICLPYESLRYEDLAMRNPFVAGWGTTAFNGPSSAVLREVQLPIWGHEPCRQAYEKDLNITNVYMCAGYADGGKDACQGDSGGPMMLPDKSGNFYLVGIVSFGKKCALPGFPGVYTKVTEFLDWIAVNMV

SEQ ID NO: 21 - DNA, 1128 bp, Limulus polyphemus
atgttggtgaataacatgttttcattgctgtgtttctcactcctgatgtctatgtttagctgcagtagtctcggcagacagcgtagacagtttgttttccccgatgatgaagaatcatgctcaaaccgatttactaacgatggaatatgtaaagatgttttgaattgtagagatcttttacaaaaaaatgattataatttactgaaagaatcaatatgcggttttgaaggcataacacccaaagtttgttgtccgaaacaaagtattgtaaatccaataacagaagcacctccaaaaactactacaactgaacgaccgccaatacggataccatccaatcttcctaaacagtgtggaaatcgtaatattacaactaccaggattattggagggcaggaagcaacacctggagcctggccctggatggctgctgtctatatcaaacaaggaggaatcagaagtgttcagtgtggaggtgcgcttgtcaccaacaggcacgtgattacagcatcgcactgtgttgtaaacagtttaggaacagatgtgatgcgagctgacgtattctcggttcgcctaggtgaacacaatttatatagcaccaatgacagttcagatccaattgattttgcagttacgtcagtgaaacatcatgaaaactttgtgctcgcgacgtatttgaatgatatcgcaattctgaagttaaacgacactgttacgtttacgcacaaaattaaaccaatttgtctaccttatgaaagcttaaggtatgaggatctagcaatgagaaacccatttgtcgccggatggggaacaacagcatttaatggcccatctagtgcagtattacgagaagtgcagttaccaatatggggacacgagccctgcaggcaggcctacgagaaggatttaaatattacaaacgtgtgtatgtgtgctgggtatgcagatggcggtaaagatgcttgccagggtgattctggaggtccaatgatgttgcctgataaaagcgggaacttttatctcgttggaattgtgtctttcggaaagaaatgcgcgttgcctggatttcctggggtttacacgaaagtgaccgaatttttagattggattgcagtaaatatggtgtag

SEQ ID NO: 22 - protein, 375 aa, Limulus polyphemus
MLVNNMFSLLCFSLLMSMFSCSSLGRQRRQFVFPDDEESCSNRFTNDGICKDVLNCRDLLQKNDYNLLKESICGFEGITPKVCCPKQSIVNPITEAPPKTTTTERPPIRIPSNLPKQCGNRNITTTRIIGGQEATPGAWPWMAAVYIKQGGIRSVQCGGALVTNRHVITASHCVVNSLGTDVMRADVFSVRLGEHNLYSTNDSSDPIDFAVTSVKHHENFVLATYLNDIAILKLNDTVTFTHKIKPICLPYESLRYEDLAMRNPFVAGWGTTAFNGPSSAVLREVQLPIWGHEPCRQAYEKDLNITNVCMCAGYADGGKDACQGDSGGPMMLPDKSGNFYLVGIVSFGKKCALPGFPGVYTKVTEFLDWIAVNMV

SEQ ID NO: 23 - protein, 4 aa, Artificial Sequence
  peptide
IEGR

SEQ ID NO: 24 - DNA, 35 bp, Artificial Sequence
  primer
ctgcaggaattcgattttttttttttttttttttt

SEQ ID NO: 25 - DNA, 35 bp, Artificial Sequence
  primer
atcgataagcttgatgatctgggcttgtgtgatga

SEQ ID NO: 26 - DNA, 15 bp, Artificial Sequence
  primer
ctgcaggaattcgat

SEQ ID NO: 27 - DNA, 15 bp, Artificial Sequence
  primer
ctacaccaagttcca

SEQ ID NO: 28 - DNA, 25 bp, Artificial Sequence
  primer
gtaaaccatgtgacaaactggaggc

SEQ ID NO: 29 - DNA, 25 bp, Artificial Sequence
  primer
aataaggcctccatcgatagaagta

SEQ ID NO: 30 - DNA, 39 bp, Artificial Sequence
  primer
ggggaattcaagcttgccaccatggtactagcgtcgttc

SEQ ID NO: 31 - DNA, 35 bp, Artificial Sequence
  primer
gggctcgagtcaaatgaactgccgaatccacgata

SEQ ID NO: 32 - DNA, 35 bp, Artificial Sequence
  primer
atcgataagcttgatcacatgcaaggaaaagttct

SEQ ID NO: 33 - DNA, 35 bp, Artificial Sequence
  primer
ctgcaggaattcgatcactgtttaaacaaactgaa

SEQ ID NO: 34 - DNA, 35 bp, Artificial Sequence
  primer
atcgataagcttgatagaccagagtggtctttctg